European Patent Application EP 4 524 249 A1, published March 19, 2025. Title: Chimeric envelope proteins of RNA virus and RNA virus vectors having the same. Applicant: ときわバイオ株式会社. Application JP. The sequence listing filed with the application follows.

SEQUENCE LISTING (51 sequences)

SEQ ID NO: 1 - DNA, 1662 bp, synthetic construct
  misc_feature 1..1662: note = Codon optimized cDNA encoding F protein of Measles virus Edmonston strain
  source 1..1662: mol_type = other DNA
atgtccatcatgggcctgaaggtgaacgtgtctgccatcttcatggccgtgctgctgaccctgcagaccccaacaggccagatccactggggcaatctgtctaagatcggagtggtgggaatcggatccgcctcttataaagtgatgacacggagctcccaccagtccctggtcatcaagctgatgcccaacatcaccctgctgaacaattgcaccagagtggagatcgccgagtaccggagactgctgaggaccgtgctggagcctatcagggacgccctgaacgccatgacacagaatatccggccagtgcagagcgtggcctctagcaggcgccacaagagatttgccggcgtggtgctggcaggagcagcactgggagtggcaaccgccgcccagatcacagccggcatcgccctgcaccagagcatgctgaactcccaggccatcgataatctgagggcctccctggagaccacaaaccaggcaatcgaggcaatcaggcaggcaggacaggagatgatcctggccgtgcagggcgtgcaggactacatcaacaatgagctgatcccctccatgaatcagctgtcttgcgatctgatcggccagaagctgggcctgaagctgctgcggtactataccgagatcctgagcctgttcggcccctccctgagagaccctatctctgccgagatcagcatccaggcactgagctatgccctgggaggcgacatcaacaaggtgctggagaagctgggatacagcggaggcgatctgctgggcatcctggagagccggggcatcaaggccagaatcacccacgtggatacagagtcctattttatcgtgctgtctatcgcctaccctaccctgagcgagatcaagggcgtgatcgtgcacaggctggagggcgtgtcttataatatcggcagccaggagtggtacaccacagtgcccaagtatgtggccacccagggctacctgatctccaacttcgacgagtcctcttgtacctttatgcctgagggcacagtgtgcagccagaatgccctgtacccaatgtccccactgctgcaggagtgtctgaggggctccaccaagtcttgcgccagaacactggtgagcggctccttcggcaaccgctttatcctgtctcagggcaacctgatcgccaattgtgccagcatcctgtgtaagtgctataccacaggcaccatcatcaaccaggacccagataagatcctgacatacatcgcagcagaccactgcccagtggtggaagtgaatggcgtgaccatccaagtgggcagccggagataccctgacgccgtgtatctgcacaggatcgatctgggaccacctatctccctggagaggctggatgtgggcacaaacctgggcaatgccatcgccaagctggaggacgccaaggagctgctggagagctccgatcagatcctgagatctatgaagggcctgtctagcaccagcatcgtgtatatcctgatcgccgtgtgtctgggaggactgatcggaatcccagcactgatctgctgttgcaggggccgctgcaacaagaagggagagcaagtgggaatgtccaggcctggcctgaagccagatctgaccggcacatctaagagctacgtgcgctctctgtga

SEQ ID NO: 2 - DNA, 1572 bp, synthetic construct
  misc_feature 1..1572: note = Codon optimized cDNA encoding C-terminal 30 aa truncated F protein of Measles virus edmonston strain
  source 1..1572: mol_type = other DNA
atgagtattatggggctgaaggtcaatgtgagcgcaatctttatggccgtgctgctgacactgcagactcctacaggacagatccactggggcaacctgtctaaaattggagtggtgggaattggatccgcctcttataaagtgatgacccggagctcccaccagtccctggtcatcaagctgatgccaaatatcaccctgctgaacaattgcacaagagtggagatcgccgagtatcggagactgctgagaaccgtgctggagccaatcagagacgccctgaacgccatgacacagaatatcagacccgtgcagtctgtggcctctagcaggcgccacaagcggttcgcaggagtggtgctggcaggagccgccctgggagtggcaaccgccgcccagatcacagccggcatcgccctgcaccagtccatgctgaactctcaggccatcgataatctgcgggcctccctggagaccacaaaccaggccatcgaggccatcagacaggccggccaggagatgatcctggccgtgcagggcgtgcaggactatatcaacaatgagctgatcccctctatgaatcagctgagctgtgatctgatcggccagaagctgggcctgaagctgctgaggtactataccgagatcctgtccctgttcggcccttctctgcgcgacccaatcagcgccgagatctccattcaggccctgagctatgcactgggcggcgacatcaacaaggtgctggagaagctgggctactctggcggcgatctgctgggcatcctggagagcaggggcatcaaggcccgcatcacccacgtggatacagagtcttacttcatcgtgctgagcatcgcctaccctacactgagcgagatcaagggcgtgatcgtgcacaggctggagggcgtgagctataatatcggctcccaggagtggtacaccacagtgcctaagtatgtggccacccagggctacctgatctccaacttcgacgagtcctcttgcacctttatgccagagggcaccgtgtgctcccagaatgccctgtacccaatgtctcccctgctgcaggagtgcctgaggggctctaccaagagctgtgcacgcacactggtgagcggatccttcggcaaccgctttatcctgtcccagggcaacctgatcgccaattgcgcctctatcctgtgcaagtgttataccacaggcaccatcatcaaccaggaccccgataagatcctgacatacatcgccgccgaccactgtcctgtggtggaagtgaatggcgtgaccatccaagtgggcagccggagataccctgacgccgtgtatctgcaccggatcgatctgggccctcccatctccctggagagactggatgtgggcacaaacctgggcaatgccatcgccaagctggaggacgccaaggagctgctggagagctccgatcagatcctgcggagcatgaagggcctgtctagcacctccatcgtgtatatcctgatcgccgtgtgcctgggcgggctgattgggattcctgctctgatttgctgctgtcgggggcggtga

SEQ ID NO: 3 - DNA, 1692 bp, synthetic construct
  misc_feature 1..1692: note = cDNA encording MeV/SeV F #2 chimeric F protein comprising C-terminal 33 aa truncated F protein of Measles virus Edmonston strain fused to C-terminal 42 aa of F protein of Sendai virus Z strain
  source 1..1692: mol_type = other DNA
atgtctatcatgggcctgaaggtgaacgtgagcgccatcttcatggccgtgctgctgaccctgcagacccctacaggccagatccactggggcaatctgtccaagatcggagtggtgggaatcggatccgcctcttataaagtgatgacaaggagctcccaccagtctctggtcatcaagctgatgccaaacatcaccctgctgaacaattgcaccagagtggagatcgccgagtaccggagactgctgcggaccgtgctggagcctatcagagacgccctgaacgccatgacacagaatatcaggccagtgcagagcgtggcctctagcaggcgccacaagaggtttgcaggagtggtgctggcaggagcagcactgggagtggcaaccgccgcccagatcacagccggcatcgccctgcaccagtccatgctgaactctcaggccatcgataatctgcgggcctccctggagaccacaaaccaggccatcgaggccatcagacaggccggccaggagatgatcctggccgtgcagggcgtgcaggactatatcaacaatgagctgatcccctctatgaatcagctgagctgcgatctgatcggccagaagctgggcctgaagctgctgaggtactataccgagatcctgtccctgttcggcccttctctgcgcgacccaatcagcgccgagatctccatccaggcactgagctatgccctgggaggcgacatcaacaaggtgctggagaagctgggatactccggaggcgatctgctgggcatcctggagtctaggggcatcaaggcccgcatcacccacgtggatacagagtcttattttatcgtgctgagcatcgcctaccctacactgagcgagatcaagggcgtgatcgtgcacaggctggagggcgtgagctataatatcggctcccaggagtggtacaccacagtgcccaagtatgtggccacccagggctacctgatctccaacttcgacgagtcctcttgtacctttatgcctgagggcacagtgtgctcccagaatgccctgtacccaatgtctcccctgctgcaggagtgtctgaggggctctaccaagagctgcgcacgcacactggtgagcggatccttcggcaaccggttcatcctgagccagggcaacctgatcgccaattgtgcctccatcctgtgtaagtgctataccacaggcaccatcatcaaccaggacccagataagatcctgacatacatcgcagcagaccactgcccagtggtggaagtgaatggcgtgaccatccaagtgggctctcggagataccccgacgccgtgtatctgcaccggatcgatctgggcccccctatcagcctggagagactggatgtgggcacaaacctgggcaatgccatcgccaagctggaggacgccaaggagctgctggagagctccgatcagatcctgcggagcatgaagggcctgtctagcacctccatcgtgtatatcctgatcgccgtgtgtctgggaggactgatcggaatcccagcactgatctgctgttgcagactgaggcgctccatgctgatgggcaaccccgacgatcggatccctagagacacctatacactggagcccaagatccggcacatgtataccaatggcggcttcgatgccatggccgagaagagatgatga

SEQ ID NO: 4 - DNA, 1674 bp, synthetic construct
  misc_feature 1..1674: note = cDNA encoding MeV/Sev F #1 chimeric F protein comprising C-terminal 62 aa truncated F protein of Measles virus Edmonston strain fused to C-terminal 65 aa of F protein of Sendai virus Z strain
  source 1..1674: mol_type = other DNA
atgtccatcatgggcctgaaggtgaacgtgtctgccatcttcatggccgtgctgctgaccctgcagaccccaacaggccagatccactggggcaatctgagcaagatcggcgtggtgggcatcggctctgccagctataaagtgatgacaaggagctcccaccagtccctggtcatcaagctgatgcccaacatcaccctgctgaacaattgcacacgcgtggagatcgccgagtaccggagactgctgcggaccgtgctggagcctatcagagacgccctgaacgccatgacacagaatatcaggccagtgcagagcgtggcctctagcaggcgccacaagaggtttgcaggagtggtgctggcaggagcagcactgggagtggcaaccgccgcccagatcacagccggcatcgccctgcaccagtctatgctgaacagccaggccatcgataatctgcgggcctccctggagaccacaaaccaggccatcgaggccatcagacaggccggccaggagatgatcctggccgtgcagggcgtgcaggactatatcaacaatgagctgatccccagcatgaatcagctgtcctgtgatctgatcggccagaagctgggcctgaagctgctgaggtactataccgagatcctgtctctgttcggacctagcctgagggacccaatctccgccgagatctctatccaggcactgagctatgccctgggaggcgacatcaacaaggtgctggagaagctgggatacagcggaggcgatctgctgggcatcctggagtccaggggcatcaaggcccgcatcacccacgtggatacagagagctattttatcgtgctgtccatcgcctaccctaccctgagcgagatcaagggcgtgatcgtgcacaggctggagggcgtgtcctataatatcggctctcaggagtggtacaccacagtgcccaagtatgtggccacacagggctacctgatctccaacttcgacgagtcctcttgcacctttatgcctgagggcacagtgtgttctcagaatgccctgtacccaatgagcccactgctgcaggagtgcctgaggggcagcaccaagtcctgtgcccgcacactggtgtccggctctttcggcaaccggttcatcctgagccagggcaacctgatcgccaattgcgccagcatcctgtgcaagtgttataccacaggcaccatcatcaaccaggacccagataagatcctgacatacatcgcagcagaccactgtccagtggtggaagtgaatggcgtgaccatccaagtgggctcccggagataccctgacgccgtgtatctgcaccggatcgatctgggcccccctatctctctggagagactggatgtgggcaccaacctgggcaatgccatcgccaagctggaggacgccaaggagctgctggagagctccgatcagatcctgcggtctatgaaagtgatcacaatcatcgtggtcatggtggtcatcctggtggtcatcatcgtgatcatcatcgtgctgtaccggctgaggcgctccatgctgatgggcaaccccgacgatcggatccctagagacacctatacactggagccaaagatccggcacatgtataccaatggcggcttcgatgccatggccgagaagagatgatga

SEQ ID NO: 5 - DNA, 1698 bp, synthetic construct
  misc_feature 1..1698: note = Codon optimized cDNA encoding modified F protein of Sendai virus Z strain
  source 1..1698: mol_type = other DNA
atgacggcgtatatccagcggagccagtgcatctcgacttcactcctcgtggtactgacgacgttggtgtcctgtcagatcccgagggaccggctctccaacattggtgtgatcgtggacgaggggaagtcgttgaaaattgcgggctcgcatgaatcgaggtatatcgtcttgtcgcttgtccccggagtggatttcgagaatggttgtgggacagcgcaagtgatccagtacaaatccttgttgaaccgactccttattcccttgagggatgctttggacttgcaagaggcccttatcactgtaacgaacgatactacgcagaacgctgggaggaggcagaaacggttctttggagcggtgatcggcaccatcgcgcttggtgtggcgacgtcggcacagatcacagcgggcattgcgctggcagaagccagagaggcgaagagggacattgcactcatcaaagaaagcatgaccaagacacacaagtcgattgagttgcttcaaaatgccgtgggcgaacaaattcttgctctcaaaacgctgcaagatttcgtaaacgatgaaatcaaacctgccatcagcgaattgggttgtgagacagcggcactgagacttgggatcaagctgactcagcattatagcgagttgctgaccgccttcgggagcaattttggaacaattggggagaagtcgctcacgctccaggcgttgtcatccttgtactcagcgaacatcacagagatcatgactacaattcggacggggcagagcaacatctacgacgtcatctacaccgaacagatcaagggaactgtaattgatgtagacttggaacgatatatggtcacattgtccgtgaaaatcccgatcttgtcagaagtccctggtgtactcattcacaaggccagctcgatctcatacaacattgacggggaggaatggtacgtcaccgtgccctcgcacatcctttcgcgggcatcatttcttggaggagctgacatcaccgattgcgtggagtcacggcttacatacatctgcccacgggacccagcgcagttgatccctgactcccagcaaaaatgtattcttggggatacgacacgctgccctgtcacgaaggtagtcgattcactgattcccaagtttgcatttgtcaacggcggagtcgtagccaactgcatcgcttccacatgcacgtgcggaacgggaaggaggcccatctcgcaagaccgctcaaaaggagtcgtgtttttgacgcacgataactgtgggcttattggggtgaatggagtggagctttatgcaaatcgcagggggcatgacgccacgtggggagtccaaaatctcactgtcggacccgcgattgcgattcgcccggtggacatttcgctcaatctggccgacgcgactaacttccttcaagattccaaggccgaattggagaaggcgcgaaagatcctgtcggaagtcggccgatggtacaattcgagggagactgtaattacgatcatcgtggtgatggtcgtgattctggtcgtcatcatcgtaatcattatcgtactttaccgcctccgccgctcaatgctcatggggaatccagacgatagaatcccgagagatacatatacacttgagccgaaaattcgacacatgtataccaatgggggattcgacgcgatggccgagaaaagatga

SEQ ID NO: 6 - DNA, 1854 bp, synthetic construct
  misc_feature 1..1854: note = Codon optimized cDNA encoding H protein of Measles virus Edmonston strain
  source 1..1854: mol_type = other DNA
atgtctccccagagggaccgcatcaacgccttttacaaggataatcctcacccaaagggcagccggatcgtgatcaacagagagcacctgatgatcgatcggccttatgtgctgctggccgtgctgttcgtgatgtttctgtccctgatcggactgctggcaatcgcaggaatcaggctgcacagagccgccatctacaccgccgagatccacaagtctctgagcaccaacctggacgtgacaaatagcatcgagcaccaggtgaaggatgtgctgacacctctgttcaagatcatcggcgacgaagtgggactgaggaccccacagcgctttacagacctggtgaagttcatctccgataagatcaagtttctgaaccctgatagggagtatgacttccgcgatctgacctggtgcatcaatccccctgagaggatcaagctggactacgatcagtattgtgccgacgtggccgccgaggagctgatgaacgccctggtgaatagcaccctgctggagacacgcaccacaaaccagtttctggccgtgtccaagggcaattgctctggcccaaccacaatccggggccagttctctaacatgtccctgtctctgctggatctgtacctgggcagaggctataatgtgagctccatcgtgaccatgacaagccagggcatgtacggcggcacctatctggtggagaagccaaatctgtctagcaagcggagcgagctgtcccagctgtctatgtaccgggtgtttgaagtgggcgtgatcagaaaccccggcctgggagcacctgtgttccacatgaccaattatctggagcagcccgtgagcaacgatctgtccaattgcatggtggcactgggagagctgaagctggcagcactgtgtcacggagaggacagcatcacaatcccataccagggcagcggcaagggcgtgtccttccagctggtgaagctgggcgtgtggaagtcccccaccgacatgcagtcttgggtgccactgagcacagacgatcccgtgatcgataggctgtatctgtcctctcacaggggcgtgatcgcagacaaccaggcaaagtgggccgtgcctaccacacggaccgacgataagctgagaatggagacatgctttcagcaggcctgtaagggcaagatccaggcactgtgcgagaacccagagtgggcacctctgaaggataatagaatcccttcctacggcgtgctgtctgtggacctgagcctgaccgtggagctgaagatcaagatcgcctctggcttcggcccactgatcacacacggctccggcatggacctgtataagtctaaccacaacaacgtgtactggctgaccatcccacccatgaagaacctggccctgggcgtgatcaatacactggagtggatccctaggtttaaggtgtccccatacctgttcaacgtgcccatcaaggaggcaggagaggactgtcacgcaccaacctatctgcccgccgaggtggacggcgatgtgaagctgagctccaacctggtcatcctgcccggccaggacctgcagtacgtgctggccacctatgatacaagccgcgtggagcacgccgtggtgtactatgtgtactccccctccaggtctttcagctacttttatcctttccgcctgccaatcaagggcgtgcctatcgagctgcaggtggagtgctttacctgggatcagaagctgtggtgccggcacttctgtgtgctggcagactccgagtctggaggacacatcacccacagcggcatggtgggcatgggcgtgtcctgtaccgtgacaagagaggacggcacaaaccggagatga

SEQ ID NO: 7 - DNA, 1800 bp, synthetic construct
  misc_feature 1..1800: note = Codon opimized cDNA encoding N-terminal 18 aa truncated H protein of Measles virus Edmonston strain
  source 1..1800: mol_type = other DNA
atggggagtagaattgtgattaaccgagagcacctgatgattgaccgaccttatgtcctgctggctgtcctgtttgtgatgttcctgtctctgattggactgctggcaattgcaggaatcagactgcacagagccgccatctacaccgccgagatccacaagtctctgagcaccaacctggacgtgacaaattccatcgagcaccaggtgaaggatgtgctgacaccactgtttaagattattggcgacgaagtgggactgaggacccctcagcggttcaccgacctggtgaagttcatctctgataagatcaagtttctgaaccccgatcgggagtatgacttcagagatctgacctggtgcatcaatccccctgagcggatcaagctggactacgatcagtattgtgccgacgtggccgccgaggagctgatgaacgccctggtgaatagcaccctgctggagacaagaaccacaaaccagtttctggccgtgtccaagggcaattgctctggccctaccacaatcaggggccagttctccaacatgtccctgtctctgctggatctgtacctgggccgcggctataatgtgagctccatcgtgaccatgacatctcagggcatgtacggcggcacctatctggtggagaagcctaacctgtctagcaagagaagcgagctgtcccagctgtctatgtaccgggtgttcgaagtgggcgtgatcagaaaccctggactgggagccccagtgttccacatgaccaattatctggagcagccagtgagcaatgatctgtccaattgcatggtggccctgggagagctgaagctggccgccctgtgccacggcgaggactctatcacaattccttaccagggatctggcaagggcgtgtccttccagctggtgaagctgggcgtgtggaagagccctaccgacatgcagtcttgggtgcccctgagcacagacgatcctgtgatcgatcggctgtatctgtcctctcacagaggcgtgatcgcagacaaccaggcaaagtgggccgtgcccaccacaaggaccgacgataagctgcgcatggagacatgctttcagcaggcctgtaagggcaagatccaggccctgtgcgagaaccctgagtgggccccactgaaggataatcggatcccaagctacggcgtgctgtctgtggacctgagcctgaccgtggagctgaagatcaagatcgcctccggcttcggccccctgatcacacacggctccggcatggacctgtataagtctaatcacaacaacgtgtactggctgaccatcccacccatgaagaacctggccctgggcgtgatcaatacactggagtggatcccacggtttaaggtgtccccctacctgttcaacgtgcctatcaaggaggcaggagaggactgtcacgcaccaacctatctgcctgcagaggtggacggcgatgtgaagctgagctccaacctggtcatcctgcctggacaggacctgcagtacgtgctggccacctatgatacaagcagggtggagcacgccgtggtgtactacgtgtactccccttcccggtctttcagctacttttatccattcagactgcccatcaagggcgtgccaatcgagctgcaggtggagtgttttacctgggatcagaagctgtggtgtagacacttctgcgtgctggcagactctgagtctggcggccacatcacacactccggcatggtcggaatgggcgtgagttgcacagtgacaagggaagatggcacaaacaggcggtaa

SEQ ID NO: 8 - DNA, 1860 bp, synthetic construct
  misc_feature 1..1860: note = cDNA encoding MeV/SeV H #2 chimeric H protein comprising N-terminal 35 aa of HN protein of Sendai virus Z strain fused to N-terminal 34 aa truncated H protein of Measles virus Edmonston strain
  source 1..1860: mol_type = other DNA
atggacggcgataggggcaagcgcgacagctactggtccacctctccaagcggctccaccacaaagccagcaagcggatgggagagaagctccaaggccgacacaccctatgtgctgctggccgtgctgttcgtgatgtttctgtccctgatcggactgctggcaatcgcaggaatcaggctgcacagagccgccatctacaccgccgagatccacaagtctctgagcaccaacctggacgtgacaaatagcatcgagcaccaggtgaaggatgtgctgacacctctgtttaagatcatcggcgacgaagtgggactgaggaccccacagcgctttacagacctggtgaagttcatctccgataagatcaagtttctgaacccagatcgggagtatgacttcagagatctgacctggtgcatcaatccccctgagcggatcaagctggactacgatcagtattgtgccgacgtggccgccgaggagctgatgaacgccctggtgaatagcaccctgctggagacaagaaccacaaaccagtttctggccgtgtccaagggcaattgctctggccccaccacaatcaggggccagttctctaacatgtccctgtctctgctggatctgtacctgggccgcggctataatgtgtctagcatcgtgaccatgacaagccagggcatgtacggcggcacctatctggtggagaagcccaacctgtcctctaagaggagcgagctgtcccagctgtctatgtaccgggtgtttgaagtgggcgtgatccgcaaccctggcctgggagccccagtgttccacatgaccaattatctggagcagcctgtgagcaatgatctgtccaattgcatggtggcactgggagagctgaagctggcagcactgtgtcacggagaggacagcatcacaatcccataccagggcagcggcaagggcgtgtccttccagctggtgaagctgggcgtgtggaagtcccccaccgacatgcagtcttgggtgcccctgagcacagacgatcctgtgatcgatcggctgtatctgagctcccacagaggcgtgatcgcagacaaccaggcaaagtgggccgtgcctaccacaaggaccgacgataagctgcgcatggagacatgctttcagcaggcctgtaagggcaagatccaggcactgtgcgagaaccctgagtgggcaccactgaaggataatcgcatcccttcctacggcgtgctgtctgtggacctgagcctgaccgtggagctgaagatcaagatcgcctctggcttcggcccactgatcacacacggctccggcatggacctgtataagtctaaccacaacaacgtgtactggctgaccatcccacccatgaagaacctggccctgggcgtgatcaatacactggagtggatcccacggtttaaggtgtccccctacctgttcaacgtgcctatcaaggaggcaggagaggactgtcacgcaccaacctatctgcctgccgaggtggacggcgatgtgaagctgtctagcaacctggtcatcctgcccggccaggacctgcagtacgtgctggccacctatgatacaagcagagtggagcacgccgtggtgtactatgtgtactccccctcccggtctttcagctacttttatccattcagactgcccatcaagggcgtgcctatcgagctgcaggtggagtgctttacctgggatcagaagctgtggtgcaggcacttctgtgtgctggcagactccgagtctggaggacacatcacccacagcggcatggtgggcatgggcgtgtcctgtaccgtgacacgcgaggacggcacaaaccggagatgatga

SEQ ID NO: 9 - DNA, 1860 bp, synthetic construct
  misc_feature 1..1860: note = cDNA encoding chimeric H protein comprising N-terminal 60 aa of HN protein of Sendai virus Z strain fused to N-terminal 58 aa truncated H protein of Measles virus Edmonston strain
  source 1..1860: mol_type = other DNA
atggacggcgataggggcaagcgcgattcctactggtccacctctccaagcggctccaccacaaagcccgcctctggctgggagagaagctccaaggccgacacctggctgctgatcctgtcctttacacagtgggccctgtctatcgccaccgtgatcatctgcatcatcatctccgcccggctgcacagagccgccatctatacagccgagatccacaagtctctgagcaccaacctggacgtgacaaatagcatcgagcaccaggtgaaggatgtgctgacccctctgttcaagatcatcggcgacgaagtgggactgaggaccccacagcgctttacagacctggtgaagttcatctccgataagatcaagtttctgaacccagatcgggagtacgacttcagagatctgacctggtgcatcaatccccctgagcggatcaagctggactacgatcagtattgtgccgacgtggccgccgaggagctgatgaacgccctggtgaatagcaccctgctggagacaagaaccacaaaccagtttctggccgtgtccaagggcaattgttctggccccaccacaatcaggggccagttctccaacatgtccctgtctctgctggatctgtacctgggccgcggctataatgtgtctagcatcgtgaccatgacatctcagggcatgtacggcggcacctatctggtggagaagcccaacctgtcctctaagaggagcgagctgtcccagctgtctatgtaccgggtgtttgaagtgggcgtgatccgcaaccctggcctgggagccccagtgttccacatgacaaattatctggagcagcctgtgagcaatgatctgtccaattgcatggtggcactgggagagctgaagctggcagcactgtgtcacggagaggactctatcaccatcccataccagggcagcggcaagggcgtgtcctttcagctggtgaagctgggcgtgtggaagtcccccacagacatgcagtcttgggtgcccctgagcaccgacgatcctgtgatcgatcggctgtatctgagctcccacagaggcgtgatcgcagacaaccaggcaaagtgggccgtgcctaccacaaggacagacgataagctgcgcatggagacctgctttcagcaggcctgtaagggcaagatccaggcactgtgcgagaaccctgagtgggcaccactgaaggataatcgcatccctagctacggcgtgctgtctgtggacctgagcctgacagtggagctgaagatcaagatcgcctccggcttcggcccactgatcacccacggcagcggcatggacctgtataagtccaatcacaacaatgtgtattggctgacaatcccacccatgaagaacctggccctgggcgtgatcaataccctggagtggatcccacggtttaaggtgtccccctacctgttcaacgtgcctatcaaggaggcaggagaggactgtcacgcaccaacatatctgcctgccgaggtggacggcgatgtgaagctgtctagcaacctggtcatcctgcccggccaggacctgcagtacgtgctggccacctatgatacaagcagagtggagcacgccgtggtgtactatgtgtactccccctcccggtctttcagctacttttatccattcagactgcccatcaagggcgtgcctatcgagctgcaggtggagtgctttacctgggatcagaagctgtggtgcaggcacttctgtgtgctggcagactccgagtctggaggacacatcacacactctggcatggtgggcatgggcgtgagctgtaccgtgacacgcgaggacggcaccaaccggagatga

SEQ ID NO: 10 - DNA, 1728 bp, synthetic construct
  misc_feature 1..1728: note = Codon optimized cDNA encoding HN protein of Sendai virus Z strain
  source 1..1728: mol_type = other DNA
atggacggggaccgaggaaagagggatagctattggtcaacaagcccctccgggagcactaccaagcctgcgtcgggatgggaaaggtcaagcaaggctgacacctggctcctgattctttcgttcacgcagtgggccttgtcgattgcgacagtcatcatctgcattatcattagcgcacgccagggttattccatgaaggagtattcgatgaccgtggaagcactgaacatgagcagccgggaagtcaaagagagcttgacttcgctcattcgacaggaggtaattgcgcgagcggtgaatatccaatcgtcagtgcagactggtatccccgtacttttgaacaaaaacagccgggatgtgatccaaatgatcgacaaatcgtgctccagacaagaactcacacagcactgcgaatcaacgattgcagtgcatcacgcggatggtatcgcgcctcttgagcctcactcattttggcgctgtccggtcggggagccgtatctttcgtcagaccccgagatttcgttgctgcctggtccttcgctcctctcgggctcaacgaccattagcgggtgtgtgaggctcccatcgctctcaattggagaagcaatctacgcctattcctcaaacctcattacccaggggtgcgccgacatcgggaagtcctaccaggtacttcagttgggatacattagcttgaacagcgatatgtttcccgatctcaacccagtggtatcgcatacttacgacatcaatgataatcgcaagtcatgcagcgtggtggcgacagggacgagaggctaccaattgtgttcgatgccgacggtggacgagagaacggactactcatccgatgggattgaggatctggtacttgacgtgctcgatcttaagggacgaacaaaatcgcacagatataggaactcggaggtggacctcgatcatcccttctcagcgctttacccgtcggtgggaaacggtatcgccacagaaggctcgcttatcttcttgggctacggaggattgaccacgccgctgcagggcgatacaaaatgccgcactcagggatgtcagcaggtgtcccaagacacatgtaacgaggcattgaagattacatggctgggagggaagcaggtcgtaagcgtgatcatccaagtaaacgattacctcagcgaaagaccaaaaatcagggtgacgacgatccctattacgcagaattatcttggagccgagggcaggttgctcaaattgggggacagagtatacatctacacacgctcaagcggatggcactcgcagctccagattggggtcctcgacgtcagccatcctctgacaatcaactggacgccccatgaggcgttgtcgaggcccggtaataaggagtgcaattggtataacaaatgtcccaaggaatgtatctcgggagtctacaccgacgcatatcccctgtcccccgatgctgcgaatgtagcaacggtcacgttgtatgccaatacgagccgcgtcaatccgacaatcatgtactcgaatacgactaacatcatcaacatgcttagaatcaaggatgtccagcttgaagctgcatacacaaccacctcatgcatcacacactttggtaaagggtattgctttcacattatcgagatcaatcaaaaatccctcaacacactccagccgatgctgttcaaaacctccatccccaagttgtgcaaggcggagtcgtga

SEQ ID NO: 11 - DNA, 55 bp, synthetic construct
  misc_feature 1..55: note = Primer #1
  source 1..55: mol_type = other DNA
ctctgcggccgcctgcaggtcgacattctcgaggtgagccccacgttctgcttca

SEQ ID NO: 12 - DNA, 40 bp, synthetic construct
  misc_feature 1..40: note = Primer #2
  source 1..40: mol_type = other DNA
atatcatatgtgtacaggctggctgcggaggaacagagaa

SEQ ID NO: 13 - DNA, 391 bp, synthetic construct
  misc_feature 1..391: note = Synthetic DNA comprising CMV IE enhancer
  source 1..391: mol_type = other DNA
gtcgacattgattattgactagttattaatagtaatcaattacggggtcattagttcatagcccatatatggagttccgcgttacataacttacggtaaatggcccgcctggctgaccgcccaacgacccccgcccattgacgtcaataatgacgtatgttcccatagtaacgccaatagggactttccattgacgtcaatgggtggagtatttacggtaaactgcccacttggcagtacatcaagtgtatcatatgccaagtacgccccctattgacgtcaatgacggtaaatggcccgcctggcattatgcccagtacatgaccttatgggactttcctacttggcagtacatctacgtattagtcatcgctattaccacatggtcgac

SEQ ID NO: 14 - DNA, 275 bp, synthetic construct
  misc_feature 1..275: note = Synthetic DNA comprising SV40 late poly(A) signal
  source 1..275: mol_type = other DNA
tgtacagcttgctcgaggatccagacatgataagatacattgatgagtttggacaaaccacaactagaatgcagtgaaaaaaatgctttatttgtgaaatttgtgatgctattgctttatttgtaaccattataagctgcaataaacaagttaacaacaacaattgcattcattttatgtttcaggttcagggggaggtgtgggaggttttttaaagcaagtaaaacctctacaaatgtggtatggctgattatgatcagccgtacggcatgcat

SEQ ID NO: 15 - DNA, 57 bp, synthetic construct
  misc_feature 1..57: note = Primer #3
  source 1..57: mol_type = other DNA
ctgttcctccgcagccagccggtaccgcttggtcgacggatccagacatgataagat

SEQ ID NO: 16 - DNA, 57 bp, synthetic construct
  misc_feature 1..57: note = Primer #4
  source 1..57: mol_type = other DNA
atcttatcatgtctggatccgtcgaccaagcggtaccggctggctgcggaggaacag

SEQ ID NO: 17 - DNA, 26 bp, synthetic construct
  misc_feature 1..26: note = Primer #5
  source 1..26: mol_type = other DNA
atcctcgaggtgagccccacgttctg

SEQ ID NO: 18 - DNA, 45 bp, synthetic construct
  misc_feature 1..45: note = Primer #6
  source 1..45: mol_type = other DNA
tagtgcggccgcttgccgtacggctgatcataatcagccatacca

SEQ ID NO: 19 - DNA, 1120 bp, synthetic construct
  misc_feature 1..1120: note = Synthetic DNA comprising tandem 4 copies of chicken globin insulator
  source 1..1120: mol_type = other DNA
gcggcccgagctcacggggacagcccccccccaaagcccccagggatgtaattacgtccctcccccgctagggggcagcagcgagccgcccggggctccgctccggtccggcgctccccccgcatccccgagccggcagcgtgcggggacagcccgggcacggggaaggtggcacgggatcgctttcctctgaacgcttctcgctgctctttgagcctgcagacacctggggggatacggggaaaaagctttaggctgaaagagagatttagaatgacgcggcccgagctcacggggacagcccccccccaaagcccccagggatgtaattacgtccctcccccgctagggggcagcagcgagccgcccggggctccgctccggtccggcgctccccccgcatccccgagccggcagcgtgcggggacagcccgggcacggggaaggtggcacgggatcgctttcctctgaacgcttctcgctgctctttgagcctgcagacacctggggggatacggggaaaaagctttaggctgaaagagagatttagaatgacgcggccgcagaacggcctgggttgcaaaggagctcacggggacagcccccccccaaagcccccagggatgtaattacgtccctcccccgctagggggcagcagcgagccgcccggggctccgctccggtccggcgctccccccgcatccccgagccggcagcgtgcggggacagcccgggcacggggaaggtggcacgggatcgctttcctctgaacgcttctcgctgctctttgagcctgcagacacctggggggatacggggaaaaagctttaggctgggccgcagaacggcctgggttgcaaaggagctcacggggacagcccccccccaaagcccccagggatgtaattacgtccctcccccgctagggggcagcagcgagccgcccggggctccgctccggtccggcgctccccccgcatccccgagccggcagcgtgcggggacagcccgggcacggggaaggtggcacgggatcgctttcctctgaacgcttctcgctgctctttgagcctgcagacacctggggggatacggggaaaaagctttaggctgggccgc

SEQ ID NO: 20 - DNA, 969 bp, synthetic construct
  misc_feature 1..969: note = Synthetic DNA comprising kanamycin resistance gene
  source 1..969: mol_type = other DNA
tcatgagattatcaaaaaggatcttcacctagatccttttaaattaaaaatgaagttttaaatcaatctaaagtatatatgagtaaacttggtctgacagttagaaaaactcatcgagcatcaaatgaaactgcaatttattcatatcaggattatcaataccatatttttgaaaaagccgtttctgtaatgaaggagaaaactcaccgaggcagttccataggatggcaagatcctggtatcggtctgcgattccgactcgtccaacatcaatacaacctattaatttcccctcgtcaaaaataaggttatcaagtgagaaatcaccatgagtgacgactgaatccggtgagaatggcaaaagtttatgcatttctttccagacttgttcaacaggccagccattacgctcgtcatcaaaatcactcgcatcaaccaaaccgttattcattcgtgattgcgcctgagcgagacgaaatacgcgatcgctgttaaaaggacaattacaaacaggaatcgaatgcaaccggcgcaggaacactgccagcgcatcaacaatattttcacctgaatcaggatattcttctaatacctggaatgctgttttcccagggatcgcagtggtgagtaaccatgcatcatcaggagtacggataaaatgcttgatggtcggaagaggcataaattccgtcagccagtttagtctgaccatctcatctgtaacatcattggcaacgctacctttgccatgtttcagaaacaactctggcgcatcgggcttcccatacaatcgatagattgtcgcacctgattgcccgacattatcgcgagcccatttatacccatataaatcagcatccatgttggaatttaatcgcggcttcgagcaagacgtttcccgttgaatatggctcatactcttcctttttcaatattattgaagcatttatcagggttattgtctcatga

SEQ ID NO: 21 - DNA, 7479 bp, synthetic construct
  misc_feature 1..7479: note = Plasmid A
  source 1..7479: mol_type = other DNA
gggcgaattaattcatggccgcgggatatcactagtgcggcccgagctcacggggacagcccccccccaaagcccccagggatgtaattacgtccctcccccgctagggggcagcagcgagccgcccggggctccgctccggtccggcgctccccccgcatccccgagccggcagcgtgcggggacagcccgggcacggggaaggtggcacgggatcgctttcctctgaacgcttctcgctgctctttgagcctgcagacacctggggggatacggggaaaaagctttaggctgaaagagagatttagaatgacgcggcccgagctcacggggacagcccccccccaaagcccccagggatgtaattacgtccctcccccgctagggggcagcagcgagccgcccggggctccgctccggtccggcgctccccccgcatccccgagccggcagcgtgcggggacagcccgggcacggggaaggtggcacgggatcgctttcctctgaacgcttctcgctgctctttgagcctgcagacacctggggggatacggggaaaaagctttaggctgaaagagagatttagaatgacgcggccgcagaacggcctgggttgcaaaggagctcacggggacagcccccccccaaagcccccagggatgtaattacgtccctcccccgctagggggcagcagcgagccgcccggggctccgctccggtccggcgctccccccgcatccccgagccggcagcgtgcggggacagcccgggcacggggaaggtggcacgggatcgctttcctctgaacgcttctcgctgctctttgagcctgcagacacctggggggatacggggaaaaagctttaggctgggccgcagaacggcctgggttgcaaaggagctcacggggacagcccccccccaaagcccccagggatgtaattacgtccctcccccgctagggggcagcagcgagccgcccggggctccgctccggtccggcgctccccccgcatccccgagccggcagcgtgcggggacagcccgggcacggggaaggtggcacgggatcgctttcctctgaacgcttctcgctgctctttgagcctgcagacacctggggggatacggggaaaaagctttaggctgggccgcttgccgtacggctgatcataatcagccataccacatttgtagaggttttacttgctttaaaaaacctcccacacctccccctgaacctgaaacataaaatgaatgcaattgttgttgttaacttgtttattgcagcttataatggttacaaataaagcaatagcatcacaaatttcacaaataaagcatttttttcactgcattctagttgtggtttgtccaaactcatcaatgtatcttatcatgtctggatccgtcgaccaagcggtaccggctggctgcggaggaacagagaagggaagatataaaccccgccggtcacacgccagaagccgaaccccgccctgccccgtcccccccgaaggcagccgtccccctgcggcagccccgaggctggagatggagaaggggacggcggcgcggcgacgcacgaaggccctccccgcccatttccttcctgccggcgccgcaccgcttcgcccgcgcccgctagagggggtgcggcggcgcctcccagatttcggctccgccagatttgggacaaaggaagtccctgcgccctctcgcacgattaccataaaaggcaatggctgcggctcgccgcgcctcgacagccgccggcgctccggggccgccgcgcccctcccccgagccctccccggcccgaggcggccccgccccgcccggcacccccacctgccgccaccccccgcccggcacggcgagccccgcgccacgccccgcacggagccccgcacccgaagccgggccgtgctcagcaactcggggaggggggtgcaggggggggttacagcccgaccgccgcgcccacaccccctgctcacccccccacgcacacaccccgcacgcagcctttgttcccctcgcagcccccccgcaccgcggggcaccgcccccggccgcgctcccctcgcgcacacgcggagcgcacaaagccccgcgccgcgcccgcagcgctcacagccgccgggcagcgcgggccgcacgcggcgctccccacgcacacacacacgcacgcaccccccgagccgctcccccccgcacaaagggccctcccggagccctttaaggctttcacgcagccacagaaaagaaacgagccgtcattaaaccaagcgctaattacagcccggaggagaagggccgtcccgcccgctcacctgtgggagtaacgcggtcagtcagagccggggcgggcggcgcgaggcggcgcggagcggggcacggggcgaaggcaacgcagcgactcccgcccgccgcgcgcttcgctttttatagggccgccgccgccgccgcctcgccataaaaggaaactttcggagcgcgccgctctgattggctgccgccgcacctctccgcctcgccccgccccgcccctcgccccgccccgccccgcctggcgcgcgccccccccccccccgcccccatcgctgcacaaaataattaaaaaataaataaatacaaaattgggggtggggaggggggggagatggggagagtgaagcagaacgtggggctcacctcgacattgattattgactagttattaatagtaatcaattacggggtcattagttcatagcccatatatggagttccgcgttacataacttacggtaaatggcccgcctggctgaccgcccaacgacccccgcccattgacgtcaataatgacgtatgttcccatagtaacgccaatagggactttccattgacgtcaatgggtggagtatttacggtaaactgcccacttggcagtacatcaagtgtatcatatgccaagtacgccccctattgacgtcaatgacggtaaatggcccgcctggcattatgcccagtacatgaccttatgggactttcctacttggcagtacatctacgtattagtcatcgctattaccacatggtcgaggtgagccccacgttctgcttcactctccccatctcccccccctccccacccccaattttgtatttatttattttttaattattttgtgcagcgatgggggcggggggggggggggcgcgcgccaggcggggcggggcggggcgaggggcggggcggggcgaggcggagaggtgcggcggcagccaatcagagcggcgcgctccgaaagtttccttttatggcgaggcggcggcggcggcggccctataaaaagcgaagcgcgcggcgggcgggagtcgctgcgttgccttcgccccgtgccccgctccgcgccgcctcgcgccgcccgccccggctctgactgaccgcgttactcccacaggtgagcgggcgggacggcccttctcctccgggctgtaattagcgcttggtttaatgacggctcgtttcttttctgtggctgcgtgaaagccttaaagggctccgggagggccctttgtgcgggggggagcggctcggggggtgcgtgcgtgtgtgtgtgcgtggggagcgccgcgtgcggcccgcgctgcccggcggctgtgagcgctgcgggcgcggcgcggggctttgtgcgctccgcgtgtgcgcgaggggagcgcggccgggggcggtgccccgcggtgcgggggggctgcgaggggaacaaaggctgcgtgcggggtgtgtgcgtgggggggtgagcagggggtgtgggcgcggcggtcgggctgtaacccccccctgcacccccctccccgagttgctgagcacggcccggcttcgggtgcggggctccgtgcggggcgtggcgcggggctcgccgtgccgggcggggggtggcggcaggtgggggtgccgggcggggcggggccgcctcgggccggggagggctcgggggaggggcgcggcggccccggagcgccggcggctgtcgaggcgcggcgagccgcagccattgccttttatggtaatcgtgcgagagggcgcagggacttcctttgtcccaaatctggcggagccgaaatctgggaggcgccgccgcaccccctctagcgggcgcgggcgaagcggtgcggcgccggcaggaaggaaatgggcggggagggccttcgtgcgtcgccgcgccgccgtccccttctccatctccagcctcggggctgccgcagggggacggctgccttcgggggggacggggcagggcggggttcggcttctggcgtgtgaccggcggggtttatatcttcccttctctgttcctccgcagccagcctgtacagcttgctcgaggatccagacatgataagatacattgatgagtttggacaaaccacaactagaatgcagtgaaaaaaatgctttatttgtgaaatttgtgatgctattgctttatttgtaaccattataagctgcaataaacaagttaacaacaacaattgcattcattttatgtttcaggttcagggggaggtgtgggaggttttttaaagcaagtaaaacctctacaaatgtggtatggctgattatgatcagccgtacggcatgcatagcttgagtattctatagtgtcacctaaatagcttggcgtaatcatggtcatagctgtttcctgtgtgaaattgttatccgctcacaattccacacaacatacgagccggaagcataaagtgtaaagcctggggtgcctaatgagtgagctaactcacattaattgcgttgcgctcactgcccgctttccagtcgggaaacctgtcgtgccagctgcattaatgaatcggccaacgcgcggggagaggcggtttgcgtattgggcgctcttccgcttcctcgctcactgactcgctgcgctcggtcgttcggctgcggcgagcggtatcagctcactcaaaggcggtaatacggttatccacagaatcaggggataacgcaggaaagaacatgtgagcaaaaggccagcaaaaggccaggaaccgtaaaaaggccgcgttgctggcgtttttccataggctccgcccccctgacgagcatcacaaaaatcgacgctcaagtcagaggtggcgaaacccgacaggactataaagataccaggcgtttccccctggaagctccctcgtgcgctctcctgttccgaccctgccgcttaccggatacctgtccgcctttctcccttcgggaagcgtggcgctttctcatagctcacgctgtaggtatctcagttcggtgtaggtcgttcgctccaagctgggctgtgtgcacgaaccccccgttcagcccgaccgctgcgccttatccggtaactatcgtcttgagtccaacccggtaagacacgacttatcgccactggcagcagccactggtaacaggattagcagagcgaggtatgtaggcggtgctacagagttcttgaagtggtggcctaactacggctacactagaaggacagtatttggtatctgcgctctgctgaagccagttaccttcggaaaaagagttggtagctcttgatccggcaaacaaaccaccgctggtagcggtggtttttttgtttgcaagcagcagattacgcgcagaaaaaaaggatctcaagaagatcctttgatcttttctacggggtctgacgctcagtggaacgaaaactcacgttaagggattttggtcatgagattatcaaaaaggatcttcacctagatccttttaaattaaaaatgaagttttaaatcaatctaaagtatatatgagtaaacttggtctgacagttagaaaaactcatcgagcatcaaatgaaactgcaatttattcatatcaggattatcaataccatatttttgaaaaagccgtttctgtaatgaaggagaaaactcaccgaggcagttccataggatggcaagatcctggtatcggtctgcgattccgactcgtccaacatcaatacaacctattaatttcccctcgtcaaaaataaggttatcaagtgagaaatcaccatgagtgacgactgaatccggtgagaatggcaaaagtttatgcatttctttccagacttgttcaacaggccagccattacgctcgtcatcaaaatcactcgcatcaaccaaaccgttattcattcgtgattgcgcctgagcgagacgaaatacgcgatcgctgttaaaaggacaattacaaacaggaatcgaatgcaaccggcgcaggaacactgccagcgcatcaacaatattttcacctgaatcaggatattcttctaatacctggaatgctgttttcccagggatcgcagtggtgagtaaccatgcatcatcaggagtacggataaaatgcttgatggtcggaagaggcataaattccgtcagccagtttagtctgaccatctcatctgtaacatcattggcaacgctacctttgccatgtttcagaaacaactctggcgcatcgggcttcccatacaatcgatagattgtcgcacctgattgcccgacattatcgcgagcccatttatacccatataaatcagcatccatgttggaatttaatcgcggcttcgagcaagacgtttcccgttgaatatggctcatactcttcctttttcaatattattgaagcatttatcagggttattgtctcatgagcggatacatatttgaatgtatttagaaaaataaacaaataggggttccgcgcacatttccccgaaaagtgccacctgtatgcggtgtgaaataccgcacagatgcgtaaggagaaaataccgcatcaggcgaaattgtaaacgttaatattttgttaaaattcgcgttaaatatttgttaaatcagctcattttttaaccaataggccgaaatcggcaaaatcccttataaatcaaaagaatagaccgagatagggttgagtgttgttccagtttggaacaagagtccactattaaagaacgtggactccaacgtcaaagggcgaaaaaccgtctatcagggcgatggcccactacgtgaaccatcacccaaatcaagttttttgcggtcgaggtgccgtaaagctctaaatcggaaccctaaagggagcccccgatttagagcttgacggggaaagccggcgaacgtggcgagaaaggaagggaagaaagcgaaaggagcgggcgctagggcgctggcaagtgtagcggtcacgctgcgcgtaaccaccacacccgccgcgcttaatgcgccgctacagggcgcgtccattcgccattcaggctgcgcaactgttgggaagggcgatcggtgcgggcctcttcgctattacgccagctggcgaaagggggatgtgctgcaaggcgattaagttgggtaacgccagggttttcccagtcacgacgttgtaaaacgacggccagtgaattgtaatacgactcactata

SEQ ID NO: 22 - DNA, 1050 bp, synthetic construct
  misc_feature 1..1050: note = Codon optimized cDNA encoding M protein of Sendai virus Clone 151
  source 1..1050: mol_type = other DNA
atggcagacatctaccgctttcccaagttctcgtatgaggacaacggaaccgtggagcctctcccgttgagaacaggtcccgacaaaaaagcgattccgcatattcggatcgtcaaggtcggggacccgcctaagcacggggtacggtatctcgatctcctcttgctcggattcttcgagacacccaagcagacgacaaatttggaatccgtgtccgatcttacggagcctacgtcgtactcaatttgcggttcgggcagcctgcccattggggtggctaagtattatggaacggatcaggagctgttgaaagcgtgtaccgaccttagaatcactgtacgcagagcggtgcgggctggagaaatgatcgtctatatggtggactcaattggagcgccccttttgccctggtcgggtaggcttcgacaggggatgatctttaatgccaacaaagtcgcgctggcaccccagtgccttccggtggataaggacatccgcttccgggtcgtatttgtgaacgggacgtcgctcggggccatcacaatctccaaaatcccgaaaaccctcgcagacttggctctgccaaatagcatcagcgtgaatctgctggtcacacttaagaccgggatctcaacagagcagaaaggggtgttgccagtgttggacgatcagggggaaaagaagctgaactttatggtacacctcggattgatcagaaggaaggtcggaaaaatctacagcgtcgaatactgcaaatcgaagatcgaaagaatgcgattgatcttctccctcggacttattggcggaatttcgttccatgtccaagtcactggtacactctcaaaaacgttcatgtcacaattggcatggaaacgggccgtctgttttcccctgatggatgtgaaccctcacatgaatatggtgatttgggcagcgtcagtggagattacgggagtagatgcggtattccagccggcgattccgagagactttaggtactacccaaacgtggtcgccaaaaacatcggccgaatcaggaagctgtgataa

SEQ ID NO: 23 - DNA, 1554 bp, synthetic construct
  misc_feature 1..1554: note = Synthetic DNA comprising EGFP gene and puromycin resistance gene
  source 1..1554: mol_type = other DNA
cccgggtaatagcccacttactcctgaatctttaattaagaaaaacttagggtgaaagcgttacaccctttcttgacaaaacctaactggtaccaccatggtgagcaagggcgaggagctgttcaccggggtggtgcccatcctggtcgagctggacggcgacgtaaacggccacaagttcagcgtgtccggcgagggcgagggcgatgccacctacggcaagctgaccctgaagttcatctgcaccaccggcaagctgcccgtgccctggcccaccctcgtgaccaccctgacctacggcgtgcagtgcttcagccgctaccccgaccacatgaagcagcacgacttcttcaagtccgccatgcccgaaggctacgtccaggagcgcaccatcttcttcaaggacgacggcaactacaagacccgcgccgaggtgaagttcgagggcgacaccctggtgaaccgcatcgagctgaagggcatcgacttcaaggaggacggcaacatcctggggcacaagctggagtacaactacaacagccacaacgtctatatcatggccgacaagcagaagaacggcatcaaggtgaacttcaagatccgccacaacatcgaggacggcagcgtgcagctcgccgaccactaccagcagaacacccccatcggcgacggccccgtgctgctgcccgacaaccactacctgagcacccagtccgccctgagcaaagaccccaacgagaagcgcgatcacatggtcctgctggagttcgtgaccgccgccgggatcactctcggcatggacgagctgtacaagtaactcgaccttcccccttttttgtcccccaacttgagttaagaaaaacttagggtgaaagcgacctctctccccagctgtatttccaaacgtaccaccatgaccgagtacaagcctaccgtgcggctggccacaagggatgacgtgcctcgggccgtgaggaccctggccgccgctttcgccgactaccccgccacaagacacaccgtggacccagacagacacatcgagagggtgaccgagctgcaggagctgttcctgaccagagtgggcctggacatcggaaaggtgtgggtggccgacgacggcgccgccgtggctgtgtggacaacccccgagtccgtggaggccggcgctgtgttcgctgagatcggacctcggatggccgagctgagcggaagcagactggccgcccagcagcagatggagggcctgctggctcctcacagacctaaggagccagcttggttcctggctaccgtgggcgtgtcccctgatcaccagggcaagggcctgggcagcgccgtggtgctgcctggagtggaggccgccgagcgcgccggagtgcctgcttttctggagaccagcgcccctcgcaacctgccattctatgagagactgggcttcaccgtgacagctgacgtggaggtgcctgagggccccagaacatggtgtatgacccggaagcctggcgcctgactcgagaggctctgttccacatatatttccactgcggccgc

SEQ ID NO: 24 - DNA, 1683 bp, synthetic construct
  misc_feature 1..1683: note = cDNA encording MeV/SeV F #2 chimeric F protein comprising C-terminal 33 aa truncated F protein of Measles virus IC-B strain fused to C-terminal 42 aa of F protein of Sendai virus Z strain
  source 1..1683: mol_type = other DNA
atggggctgaaggtcaatgtgagcgcaatctttatggccgtgctgctgacactgcagactcctacaggacagatccactggggcaacctgtctaaaattggagtggtgggaattggatccgcctcttataaagtgatgacaaggagctcccaccagtctctggtcatcaagctgatgccaaacatcaccctgctgaacaattgcaccagagtggagatcgccgagtaccggagactgctgcggaccgtgctggagcctatcagagacgccctgaacgccatgacacagaatatcaggccagtgcagagcgtggcctctagcaggcgccacaagaggtttgcaggagtggtgctggcaggagcagcactgggagtggcaaccgccgcccagatcacagccggcatcgccctgcaccagtccatgctgaactctcaggccatcgataatctgcgggcctccctggagaccacaaaccaggccatcgaggccatcagacaggccggccaggagatgatcctggccgtgcagggcgtgcaggactatatcaacaatgagctgatcccctctatgaatcagctgagctgcgatctgatcggccagaagctgggcctgaagctgctgaggtactataccgagatcctgtccctgttcggcccttctctgcgcgacccaatcagcgccgagatctccatccaggcactgagctatgccctgggaggcgacatcaacaaggtgctggagaagctgggatactccggaggcgatctgctgggcatcctggagtctaggggcatcaaggcccgcatcacccacgtggatacagagtcttattttatcgtgctgagcatcgcctaccctacactgagcgagatcaagggcgtgatcgtgcacaggctggagggcgtgagctataatatcggctcccaggagtggtacaccacagtgcccaagtatgtggccacccagggctacctgatctccaacttcgacgagtcctcttgtacctttatgcctgagggcacagtgtgctcccagaatgccctgtacccaatgtctcccctgctgcaggagtgtctgaggggctctaccaagagctgcgcacgcacactggtgagcggatccttcggcaaccggttcatcctgagccagggcaacctgatcgccaattgtgcctccatcctgtgtaagtgctataccacaggcaccatcatcaaccaggacccagataagatcctgacatacatcgcagcagaccactgcccagtggtggaagtgaatggcgtgaccatccaagtgggctctcggagataccccgacgccgtgtatctgcaccggatcgatctgggcccccctatcagcctggagagactggatgtgggcacaaacctgggcaatgccatcgccaagctggaggacgccaaggagctgctggagagctccgatcagatcctgcggagcatgaagggcctgtctagcacctccatcgtgtatatcctgatcgccgtgtgtctgggaggactgatcggaatcccagcactgatctgctgttgcagactgaggcgctccatgctgatgggcaaccccgacgatcggatccctagagacacctatacactggagcccaagatccggcacatgtataccaatggcggcttcgatgccatggccgagaagagatgatga

SEQ ID NO: 25 - DNA, 4392 bp, synthetic construct
  misc_feature 1..4392: note = cDNA inserted into SeV vector A
  source 1..4392: mol_type = other DNA
ttaagaaaaacttagggtgaaagaaatttcaccgctagcacctggtaccaccatggcagacatctaccgctttcccaagttctcgtatgaggacaacggaaccgtggagcctctcccgttgagaacaggtcccgacaaaaaagcgattccgcatattcggatcgtcaaggtcggggacccgcctaagcacggggtacggtatctcgatctcctcttgctcggattcttcgagacacccaagcagacgacaaatttggaatccgtgtccgatcttacggagcctacgtcgtactcaatttgcggttcgggcagcctgcccattggggtggctaagtattatggaacggatcaggagctgttgaaagcgtgtaccgaccttagaatcactgtacgcagagcggtgcgggctggagaaatgatcgtctatatggtggactcaattggagcgccccttttgccctggtcgggtaggcttcgacaggggatgatctttaatgccaacaaagtcgcgctggcaccccagtgccttccggtggataaggacatccgcttccgggtcgtatttgtgaacgggacgtcgctcggggccatcacaatctccaaaatcccgaaaaccctcgcagacttggctctgccaaatagcatcagcgtgaatctgctggtcacacttaagaccgggatctcaacagagcagaaaggggtgttgccagtgttggacgatcagggggaaaagaagctgaactttatggtacacctcggattgatcagaaggaaggtcggaaaaatctacagcgtcgaatactgcaaatcgaagatcgaaagaatgcgattgatcttctccctcggacttattggcggaatttcgttccatgtccaagtcactggtacactctcaaaaacgttcatgtcacaattggcatggaaacgggccgtctgttttcccctgatggatgtgaaccctcacatgaatatggtgatttgggcagcgtcagtggagattacgggagtagatgcggtattccagccggcgattccgagagactttaggtactacccaaacgtggtcgccaaaaacatcggccgaatcaggaagctgtgataagtcgaccgattaagaaaaacttagggtgaaagttcatcgcatccgcttggcgcgtacgaccatggacggcgataggggcaagcgcgattcctactggtccacctctccaagcggctccaccacaaagcccgcctctggctgggagagaagctccaaggccgacacctggctgctgatcctgtcctttacacagtgggccctgtctatcgccaccgtgatcatctgcatcatcatctccgcccggctgcacagagccgccatctatacagccgagatccacaagtctctgagcaccaacctggacgtgacaaatagcatcgagcaccaggtgaaggatgtgctgacccctctgttcaagatcatcggcgacgaagtgggactgaggaccccacagcgctttacagacctggtgaagttcatctccgataagatcaagtttctgaacccagatcgggagtacgacttcagagatctgacctggtgcatcaatccccctgagcggatcaagctggactacgatcagtattgtgccgacgtggccgccgaggagctgatgaacgccctggtgaatagcaccctgctggagacaagaaccacaaaccagtttctggccgtgtccaagggcaattgttctggccccaccacaatcaggggccagttctccaacatgtccctgtctctgctggatctgtacctgggccgcggctataatgtgtctagcatcgtgaccatgacatctcagggcatgtacggcggcacctatctggtggagaagcccaacctgtcctctaagaggagcgagctgtcccagctgtctatgtaccgggtgtttgaagtgggcgtgatccgcaaccctggcctgggagccccagtgttccacatgacaaattatctggagcagcctgtgagcaatgatctgtccaattgcatggtggcactgggagagctgaagctggcagcactgtgtcacggagaggactctatcaccatcccataccagggcagcggcaagggcgtgtcctttcagctggtgaagctgggcgtgtggaagtcccccacagacatgcagtcttgggtgcccctgagcaccgacgatcctgtgatcgatcggctgtatctgagctcccacagaggcgtgatcgcagacaaccaggcaaagtgggccgtgcctaccacaaggacagacgataagctgcgcatggagacctgctttcagcaggcctgtaagggcaagatccaggcactgtgcgagaaccctgagtgggcaccactgaaggataatcgcatccctagctacggcgtgctgtctgtggacctgagcctgacagtggagctgaagatcaagatcgcctccggcttcggcccactgatcacccacggcagcggcatggacctgtataagtccaatcacaacaatgtgtattggctgacaatcccacccatgaagaacctggccctgggcgtgatcaataccctggagtggatcccacggtttaaggtgtccccctacctgttcaacgtgcctatcaaggaggcaggagaggactgtcacgcaccaacatatctgcctgccgaggtggacggcgatgtgaagctgtctagcaacctggtcatcctgcccggccaggacctgcagtacgtgctggccacctatgatacaagcagagtggagcacgccgtggtgtactatgtgtactccccctcccggtctttcagctacttttatccattcagactgcccatcaagggcgtgcctatcgagctgcaggtggagtgctttacctgggatcagaagctgtggtgcaggcacttctgtgtgctggcagactccgagtctggaggacacatcacacactctggcatggtgggcatgggcgtgagctgtaccgtgacacgcgaggacggcaccaaccggagatgactcgagtcagagacctgcaacaatgtctcaagcagacaccacctggcagtcggagccaccgggtcactccttgtcttaaataagaaaaacttagggataaagtcccttagatctagcctggtaccaccatggtctcagtgatcaagcccgagatgaagatgaagtactttatggacggcagcgtgaacggacacgagtttacagtcgagggggaaggcaccggcaagccctatgagggccaccaggagatgaccctgcgggtgaccatggccaagggcggccccatgcctttcagcttcgacctggtgtcccacaccttctgctacggccacaggccctttacaaagtatccagaggagatcccagactacttcaagcaggccttccctgagggcctgtcctgggagagatccctgcagtttgaggatggcggctttgccgccgtgtctgcccacatcagcctgcggggcaactgctttgagcacaagagcaagtttgtgggcgtgaacttcccagccgatggcccagtgatgcagaaccagagctctgactgggagcccagcacagagaagatcaccacctgtgatggcgtgctgaagggcgatgtgaccatgtacctgaagctggccggcggcggcaaccacaagtgccagttcaagaccacctataaggccgccaagaagatcctgaagatgccccagtcccacttcatcggccacagactggtgcggaaaactgaagggaacattaccgaactggtggaagatgccgtcgcacattgctgataagtcgaccagatctgtatataataagaaaaacttagggtgaaagtgaggttgcgcggtattttagcgtacgaccatgcctctgagccaggaagaatctactctgattgaacgagccactgctactattaactccatccccatctccgaagactactccgtcgcctctgccgccctgtcctctgatggcaggatcttcacaggcgtgaacgtgtaccacttcacaggcggcccctgtgccgagctggtggtgctgggcaccgccgccgccgccgccgccggcaacctgacctgcatcgtggccatcggcaacgagaacagaggcatcctgagcccctgtggccgctgcaggcaggtgctgctggacctgcaccctggcatcaaggccatcgtgaaggacagcgatggccagccaactgctgtcggaattagagaactgctgccctcaggatacgtctgggaaggatgataactcgagtgtcggctttgctgacactagagtcatctccgaacatccacaatatctctcagtctcttacgtctctcacagtatgcggccgcttaagaaaaacccagggtgaatg

SEQ ID NO: 26 - DNA, 4224 bp, synthetic construct
  misc_feature 1..4224: note = cDNA inserted into SeV vector B
  source 1..4224: mol_type = other DNA
ttaagaaaaacttagggtgaaagaaatttcaccgctagcacctggtaccaccatggcagacatctaccgctttcccaagttctcgtatgaggacaacggaaccgtggagcctctcccgttgagaacaggtcccgacaaaaaagcgattccgcatattcggatcgtcaaggtcggggacccgcctaagcacggggtacggtatctcgatctcctcttgctcggattcttcgagacacccaagcagacgacaaatttggaatccgtgtccgatcttacggagcctacgtcgtactcaatttgcggttcgggcagcctgcccattggggtggctaagtattatggaacggatcaggagctgttgaaagcgtgtaccgaccttagaatcactgtacgcagagcggtgcgggctggagaaatgatcgtctatatggtggactcaattggagcgccccttttgccctggtcgggtaggcttcgacaggggatgatctttaatgccaacaaagtcgcgctggcaccccagtgccttccggtggataaggacatccgcttccgggtcgtatttgtgaacgggacgtcgctcggggccatcacaatctccaaaatcccgaaaaccctcgcagacttggctctgccaaatagcatcagcgtgaatctgctggtcacacttaagaccgggatctcaacagagcagaaaggggtgttgccagtgttggacgatcagggggaaaagaagctgaactttatggtacacctcggattgatcagaaggaaggtcggaaaaatctacagcgtcgaatactgcaaatcgaagatcgaaagaatgcgattgatcttctccctcggacttattggcggaatttcgttccatgtccaagtcactggtacactctcaaaaacgttcatgtcacaattggcatggaaacgggccgtctgttttcccctgatggatgtgaaccctcacatgaatatggtgatttgggcagcgtcagtggagattacgggagtagatgcggtattccagccggcgattccgagagactttaggtactacccaaacgtggtcgccaaaaacatcggccgaatcaggaagctgtgataagtcgaccgattaagaaaaacttagggtgaaagttcatcgcatccgcttggcgcgtacgaccatgtctatcatgggcctgaaggtgaacgtgagcgccatcttcatggccgtgctgctgaccctgcagacccctacaggccagatccactggggcaatctgtccaagatcggagtggtgggaatcggatccgcctcttataaagtgatgacaaggagctcccaccagtctctggtcatcaagctgatgccaaacatcaccctgctgaacaattgcaccagagtggagatcgccgagtaccggagactgctgcggaccgtgctggagcctatcagagacgccctgaacgccatgacacagaatatcaggccagtgcagagcgtggcctctagcaggcgccacaagaggtttgcaggagtggtgctggcaggagcagcactgggagtggcaaccgccgcccagatcacagccggcatcgccctgcaccagtccatgctgaactctcaggccatcgataatctgcgggcctccctggagaccacaaaccaggccatcgaggccatcagacaggccggccaggagatgatcctggccgtgcagggcgtgcaggactatatcaacaatgagctgatcccctctatgaatcagctgagctgcgatctgatcggccagaagctgggcctgaagctgctgaggtactataccgagatcctgtccctgttcggcccttctctgcgcgacccaatcagcgccgagatctccatccaggcactgagctatgccctgggaggcgacatcaacaaggtgctggagaagctgggatactccggaggcgatctgctgggcatcctggagtctaggggcatcaaggcccgcatcacccacgtggatacagagtcttattttatcgtgctgagcatcgcctaccctacactgagcgagatcaagggcgtgatcgtgcacaggctggagggcgtgagctataatatcggctcccaggagtggtacaccacagtgcccaagtatgtggccacccagggctacctgatctccaacttcgacgagtcctcttgtacctttatgcctgagggcacagtgtgctcccagaatgccctgtacccaatgtctcccctgctgcaggagtgtctgaggggctctaccaagagctgcgcacgcacactggtgagcggatccttcggcaaccggttcatcctgagccagggcaacctgatcgccaattgtgcctccatcctgtgtaagtgctataccacaggcaccatcatcaaccaggacccagataagatcctgacatacatcgcagcagaccactgcccagtggtggaagtgaatggcgtgaccatccaagtgggctctcggagataccccgacgccgtgtatctgcaccggatcgatctgggcccccctatcagcctggagagactggatgtgggcacaaacctgggcaatgccatcgccaagctggaggacgccaaggagctgctggagagctccgatcagatcctgcggagcatgaagggcctgtctagcacctccatcgtgtatatcctgatcgccgtgtgtctgggaggactgatcggaatcccagcactgatctgctgttgcagactgaggcgctccatgctgatgggcaaccccgacgatcggatccctagagacacctatacactggagcccaagatccggcacatgtataccaatggcggcttcgatgccatggccgagaagagatgatgactcgagtcagagacctgcaacaatgtctcaagcagacaccacctggcagtcggagccaccgggtcactccttgtcttaaataagaaaaacttagggataaagtcccttagatctagcctggtaccaccatggtctcagtgatcaagcccgagatgaagatgaagtactttatggacggcagcgtgaacggacacgagtttacagtcgagggggaaggcaccggcaagccctatgagggccaccaggagatgaccctgcgggtgaccatggccaagggcggccccatgcctttcagcttcgacctggtgtcccacaccttctgctacggccacaggccctttacaaagtatccagaggagatcccagactacttcaagcaggccttccctgagggcctgtcctgggagagatccctgcagtttgaggatggcggctttgccgccgtgtctgcccacatcagcctgcggggcaactgctttgagcacaagagcaagtttgtgggcgtgaacttcccagccgatggcccagtgatgcagaaccagagctctgactgggagcccagcacagagaagatcaccacctgtgatggcgtgctgaagggcgatgtgaccatgtacctgaagctggccggcggcggcaaccacaagtgccagttcaagaccacctataaggccgccaagaagatcctgaagatgccccagtcccacttcatcggccacagactggtgcggaaaactgaagggaacattaccgaactggtggaagatgccgtcgcacattgctgataagtcgaccagatctgtatataataagaaaaacttagggtgaaagtgaggttgcgcggtattttagcgtacgaccatgcctctgagccaggaagaatctactctgattgaacgagccactgctactattaactccatccccatctccgaagactactccgtcgcctctgccgccctgtcctctgatggcaggatcttcacaggcgtgaacgtgtaccacttcacaggcggcccctgtgccgagctggtggtgctgggcaccgccgccgccgccgccgccggcaacctgacctgcatcgtggccatcggcaacgagaacagaggcatcctgagcccctgtggccgctgcaggcaggtgctgctggacctgcaccctggcatcaaggccatcgtgaaggacagcgatggccagccaactgctgtcggaattagagaactgctgccctcaggatacgtctgggaaggatgataactcgagtgtcggctttgctgacactagagtcatctccgaacatccacaatatctctcagtctcttacgtctctcacagtatgcggccgcttaagaaaaacccagggtgaatg

SEQ ID NO: 27 - DNA, 2538 bp, synthetic construct
  misc_feature 1..2538: note = cDNA inserted into SeV vector C
  source 1..2538: mol_type = other DNA
ttaagaaaaacttagggtgaaagaaatttcaccgctagcacctggtaccaccatggcagacatctaccgctttcccaagttctcgtatgaggacaacggaaccgtggagcctctcccgttgagaacaggtcccgacaaaaaagcgattccgcatattcggatcgtcaaggtcggggacccgcctaagcacggggtacggtatctcgatctcctcttgctcggattcttcgagacacccaagcagacgacaaatttggaatccgtgtccgatcttacggagcctacgtcgtactcaatttgcggttcgggcagcctgcccattggggtggctaagtattatggaacggatcaggagctgttgaaagcgtgtaccgaccttagaatcactgtacgcagagcggtgcgggctggagaaatgatcgtctatatggtggactcaattggagcgccccttttgccctggtcgggtaggcttcgacaggggatgatctttaatgccaacaaagtcgcgctggcaccccagtgccttccggtggataaggacatccgcttccgggtcgtatttgtgaacgggacgtcgctcggggccatcacaatctccaaaatcccgaaaaccctcgcagacttggctctgccaaatagcatcagcgtgaatctgctggtcacacttaagaccgggatctcaacagagcagaaaggggtgttgccagtgttggacgatcagggggaaaagaagctgaactttatggtacacctcggattgatcagaaggaaggtcggaaaaatctacagcgtcgaatactgcaaatcgaagatcgaaagaatgcgattgatcttctccctcggacttattggcggaatttcgttccatgtccaagtcactggtacactctcaaaaacgttcatgtcacaattggcatggaaacgggccgtctgttttcccctgatggatgtgaaccctcacatgaatatggtgatttgggcagcgtcagtggagattacgggagtagatgcggtattccagccggcgattccgagagactttaggtactacccaaacgtggtcgccaaaaacatcggccgaatcaggaagctgtgataagtcgaccgattaagaaaaacttagggtgaaagttcatcgcatccgcttggcgcgtacgaccatgtaactcgagtcagagacctgcaacaatgtctcaagcagacaccacctggcagtcggagccaccgggtcactccttgtcttaaataagaaaaacttagggataaagtcccttagatctagcctggtaccaccatggtctcagtgatcaagcccgagatgaagatgaagtactttatggacggcagcgtgaacggacacgagtttacagtcgagggggaaggcaccggcaagccctatgagggccaccaggagatgaccctgcgggtgaccatggccaagggcggccccatgcctttcagcttcgacctggtgtcccacaccttctgctacggccacaggccctttacaaagtatccagaggagatcccagactacttcaagcaggccttccctgagggcctgtcctgggagagatccctgcagtttgaggatggcggctttgccgccgtgtctgcccacatcagcctgcggggcaactgctttgagcacaagagcaagtttgtgggcgtgaacttcccagccgatggcccagtgatgcagaaccagagctctgactgggagcccagcacagagaagatcaccacctgtgatggcgtgctgaagggcgatgtgaccatgtacctgaagctggccggcggcggcaaccacaagtgccagttcaagaccacctataaggccgccaagaagatcctgaagatgccccagtcccacttcatcggccacagactggtgcggaaaactgaagggaacattaccgaactggtggaagatgccgtcgcacattgctgataagtcgaccagatctgtatataataagaaaaacttagggtgaaagtgaggttgcgcggtattttagcgtacgaccatgcctctgagccaggaagaatctactctgattgaacgagccactgctactattaactccatccccatctccgaagactactccgtcgcctctgccgccctgtcctctgatggcaggatcttcacaggcgtgaacgtgtaccacttcacaggcggcccctgtgccgagctggtggtgctgggcaccgccgccgccgccgccgccggcaacctgacctgcatcgtggccatcggcaacgagaacagaggcatcctgagcccctgtggccgctgcaggcaggtgctgctggacctgcaccctggcatcaaggccatcgtgaaggacagcgatggccagccaactgctgtcggaattagagaactgctgccctcaggatacgtctgggaaggatgataactcgagtgtcggctttgctgacactagagtcatctccgaacatccacaatatctctcagtctcttacgtctctcacagtatgcggccgcttaagaaaaacccagggtgaatg

SEQ ID NO: 28 - DNA, 4134 bp, synthetic construct
  misc_feature 1..4134: note = cDNA inserted into SeV vector D
  source 1..4134: mol_type = other DNA
ttaagaaaaacttagggtgaaagaaatttcaccgctagcacctggtaccaccatggcaagcaaagtctatgacccagaacagcgaaaaaggatgattacaggacctcagtggtgggcacgatgcaaacagatgaatgtgctggacagcttcatcaactactatgacagcgagaagcacgccgagaatgccgtgatcttcctgcacggcaatgccgcctccagctacctgtggcgccacgtggtgcctcacatcgagccagtggcccgctgcatcatcccagacctgatcggcatgggcaagagcggcaagtccggcaacggctcctataggctgctggaccactacaagtacctgaccgcctggttcgagctgctgaacctgcccaagaagatcatcttcgtgggccacgactggggcgcctgcctggccttccactacagctacgagcaccaggacaagatcaaggccatcgtgcacgccgagagcgtggtggatgtgatcgagagctgggatgagtggccagacatcgaggaggacatcgccctgatcaagagcgaggagggcgagaagatggtgctggagaacaacttctttgtggagaccatgctgcccagcaagatcatgaggaagctggagccagaggagtttgccgcctacctggagccattcaaggagaagggcgaggtgcgcaggcccaccctgtcctggcccagggagatccccctggtgaagggcggcaagccagatgtggtgcagatcgtgcggaactacaatgcctatctgagggccagcgacgatctgcccaagatgttcatcgagtccgatcctggcttcttcagcaatgccatcgtggagggcgccaagaagttccccaatacagagtttgtgaaggtgaagggcctgcacttctcccaggaggatgccccagacgagatgggcaagtacatcaagagctttgtggagagggtgctgaagaacgagcagaacagcgcctgcaagaactggttctcctctctgagccactttgtgatccacctgaacagccacggctttcccccagaggtggaggagcaggccgccggcaccctgcccatgagctgtgcccaggaatcaggaatggatagacacccagcagcttgtgccagtgcccgaatcaacgtgtaatgagtcgaccgattaagaaaaacttagggtgaaagttcatcgcatccgcttggcgcgtacgaccatgctgggaccttgtatgctgctgctgctgctgctgctgggactgagactgcagctgtcactgggaatcatccccgtggaagaagaaaaccctgacttctggaacagggaggccgccgaggccctgggcgccgccaagaagctgcagccagcccagacagccgccaagaatctgatcatcttcctgggcgacggcatgggcgtgtctacagtgaccgccgccaggatcctgaagggccagaagaaggacaagctgggccctgagatcccactggccatggacaggtttccatatgtggccctgtctaagacctacaatgtggacaagcacgtgcccgattctggcgccaccgccacagcctacctgtgcggcgtgaagggcaatttccagaccatcggcctgtctgccgccgccaggtttaaccagtgcaacaccacacgcggcaacgaggtaatctctgtgatgaacagggccaagaaggccggcaagtctgtgggcgtggtgaccaccacaagggtgcagcacgcctccccagccggcacatatgcccacaccgtgaacagaaactggtattctgatgccgatgtgcccgcctctgccaggcaggagggctgtcaggacatcgccacccagctgatctccaacatggacatcgacgtgatcctgggcggcggcaggaagtatatgttcaggatgggcacaccagacccagagtatccagatgactactctcagggcggcacccgcctggacggcaagaacctggtgcaggagtggctggccaagcggcagggcgcccgctacgtgtggaacaggacagagctgatgcaggccagcctggatccatctgtgacccacctgatgggcctgtttgagccaggcgacatgaagtatgagatccacagggacagcaccctggacccatctctgatggagatgacagaggccgccctgaggctgctgtctagaaaccctcgcggctttttcctgttcgtggagggcggcaggatcgaccacggccaccacgagtctcgcgcctacagagccctgacagagaccatcatgttcgatgatgccatcgagcgggccggccagctgacatctgaggaggataccctgagcctggtgacagccgaccacagccacgtgttcagctttggcggctacccactgcggggctccagcatctttggcctggccccaggcaaggccagggacaggaaggcctatacagtgctgctgtatggcaacggcccaggctacgtgctgaaggatggcgccaggccagatgtgacagagtctgagtctggctccccagagtatcggcagcagtctgccgtgcccctggatgaggagacccacgccggcgaggacgtggccgtgtttgccaggggcccccaggcccacctggtgcacggcgtgcaggagcagaccttcatcgcccacgtgatggccttcgccgcctgtctggagccatacaccgcttgtgatctggctcctcctgctggcaccactgacgctgctcatcctggctgactcgagtcagagacctgcaacaatgtctcaagcagacaccacctggcagtcggagccaccgggtcactccttgtcttaaataagaaaaacttagggataaagtcccttagatctagcctggtaccaccatggtctcagtgatcaagcccgagatgaagatgaagtactttatggacggcagcgtgaacggacacgagtttacagtcgagggggaaggcaccggcaagccctatgagggccaccaggagatgaccctgcgggtgaccatggccaagggcggccccatgcctttcagcttcgacctggtgtcccacaccttctgctacggccacaggccctttacaaagtatccagaggagatcccagactacttcaagcaggccttccctgagggcctgtcctgggagagatccctgcagtttgaggatggcggctttgccgccgtgtctgcccacatcagcctgcggggcaactgctttgagcacaagagcaagtttgtgggcgtgaacttcccagccgatggcccagtgatgcagaaccagagctctgactgggagcccagcacagagaagatcaccacctgtgatggcgtgctgaagggcgatgtgaccatgtacctgaagctggccggcggcggcaaccacaagtgccagttcaagaccacctataaggccgccaagaagatcctgaagatgccccagtcccacttcatcggccacagactggtgcggaaaactgaagggaacattaccgaactggtggaagatgccgtcgcacattgctgataagtcgaccagatctgtatataataagaaaaacttagggtgaaagtgaggttgcgcggtattttagcgtacgaccatgcctctgagccaggaagaatctactctgattgaacgagccactgctactattaactccatccccatctccgaagactactccgtcgcctctgccgccctgtcctctgatggcaggatcttcacaggcgtgaacgtgtaccacttcacaggcggcccctgtgccgagctggtggtgctgggcaccgccgccgccgccgccgccggcaacctgacctgcatcgtggccatcggcaacgagaacagaggcatcctgagcccctgtggccgctgcaggcaggtgctgctggacctgcaccctggcatcaaggccatcgtgaaggacagcgatggccagccaactgctgtcggaattagagaactgctgccctcaggatacgtctgggaaggatgataactcgagtgtcggctttgctgacactagagtcatctccgaacatccacaatatctctcagtctcttacgtctctcacagtatgcggccgcttaagaaaaacccagggtgaatg

SEQ ID NO: 29 - DNA, 1086 bp, Homo sapiens
  source 1..1086: mol_type = genomic DNA
atggcgggacacctggcttcggatttcgccttctcgccccctccaggtggtggaggtgatgggccaggggggccggagccgggctgggttgatcctcggacctggctaagcttccaaggccctcctggagggccaggaatcgggccgggggttgggccaggctctgaggtgtgggggattcccccatgccccccgccgtatgagttctgtggggggatggcgtactgtgggccccaggttggagtggggctagtgccccaaggcggcttggagacctctcagcctgagggcgaagcaggagtcggggtggagagcaactccgatggggcctccccggagccctgcaccgtcacccctggtgccgtgaagctggagaaggagaagctggagcaaaacccggaggagtcccaggacatcaaagctctgcagaaagaactggagcaatttgccaagctcctgaagcagaagaggatcaccctgggatatacacaggccgatgtggggctcaccctgggggttctatttgggaaggtattcagccaaacgaccatctgccgctttgaggctctgcagcttagcttcaagaacatgtgtaagctgcggcccttgctgcagaagtgggtggaggaagctgacaacaatgaaaatcttcaggagatatgcaaagcagaaaccctcgtgcaggcccgaaagagaaagcgaaccagtatcgagaaccgagtgagaggcaacctggagaatttgttcctgcagtgcccgaaacccacactgcagcagatcagccacatcgcccagcagcttgggctggagaaggatgtggtccgagtgtggttctgtaaccggcgccagaagggcaagcgatcaagcagcgactatgcacaacgagaggattttgaggctgctgggtctcctttctcagggggaccagtgtcctttcctctggccccagggccccattttggaaccccaggctatgggagccctcacttcactgcactgtactcctcggtccctttccctgagggggaagcctttccccctgtctccgtcaccactctgggctctcccatgcattcaaactgataa

SEQ ID NO: 30 - DNA, 954 bp, Homo sapiens
  source 1..954: mol_type = genomic DNA
atgtataacatgatggagacggagctgaagccgccgggcccgcagcaaacttcggggggcggcggcggcaactccaccgcggcggcggccggcggcaaccagaaaaacagcccggaccgcgtcaagcggcccatgaatgccttcatggtgtggtcccgcgggcagcggcgcaagatggcccaggagaaccccaagatgcacaactcggagatcagcaagcgcctgggcgccgagtggaaacttttgtcggagacggagaagcggccgttcatcgacgaggctaagcggctgcgagcgctgcacatgaaggagcacccggattataaataccggccccggcggaaaaccaagacgctcatgaagaaggataagtacacgctgcccggcgggctgctggcccccggcggcaatagcatggcgagcggggtcggggtgggcgccggcctgggcgcgggcgtgaaccagcgcatggacagttacgcgcacatgaacggctggagcaacggcagctacagcatgatgcaggaccagctgggctacccgcagcaccctggcctcaatgcgcacggcgcagcgcagatgcagcccatgcaccgctacgacgtgagcgccctgcagtacaactccatgaccagctcgcagacctacatgaacggctcgcccacctacagcatgtcctactcgcagcagggcacccctggcatggctcttggctccatgggttcggtggtcaagtccgaggccagctccagcccccctgtggttacctcttcctcccactccagggcgccctgccaggccggggacctccgggacatgatcagcatgtatctccccggcgccgaggtgccggaacccgccgcccccagcagacttcacatgtcccagcactaccagagcggcccggtgcccggcacggccattaacggcacactgcccctctcacacatgtga

SEQ ID NO: 31 - DNA, 1440 bp, Homo sapiens
  source 1..1440: mol_type = genomic DNA
atgaggcagccacctggcgagtctgacatggctgtcagcgacgcgctgctcccatctttctccacgttcgcgtctggcccggcgggaagggagaagacactgcgtcaagcaggtgccccgaataaccgctggcgggaggagctctcccacatgaagcgacttcccccagtgcttcccggccgcccctatgacctggcggcggcgaccgtggccacagacctggagagcggcggagccggtgcggcttgcggcggtagcaacctggcgcccctacctcggagagagaccgaggagttcaacgatctcctggacctggactttattctctccaattcgctgacccatcctccggagtcagtggccgccaccgtgtcctcgtcagcgtcagcctcctcttcgtcgtcgccgtcgagcagcggccctgccagcgcgccctccacctgcagcttcacctatccgatccgggccgggaacgaccctggcgtggcgccgggcggcacgggcggaggcctcctctatggcagggagtccgctccccctccgacggctcccttcaacctggcggacatcaacgacgtgagcccctcgggcggcttcgtggccgagctcctgcggccagaattggacccggtctacattccgccgcagcagccgcagccgccaggtggcgggctgatgggcaagttcgtgctgaaggcgtcgctgagcgcccctggcagcgagtacggcagcccgtcggtcatcagcgtcagcaaaggcagccctgacggcagccacccggtggtggtggcgccctacaacggcgggccgccgcgcacgtgccccaagatcaagcaggaggcggtctcttcgtgcacccacttgggcgctggaccccctctcagcaatggccaccggccggctgcacacgacttccccctggggcggcagctccccagcaggactaccccgaccctgggtcttgaggaagtgctgagcagcagggactgtcaccctgccctgccgcttcctcccggcttccatccccatccggggcccaattacccatccttcctgcccgatcagatgcagccgcaagtcccgccgctccattaccaagagctcatgccacccggttcctgcatgccagaggagcccaagccaaagaggggaagacgatcgtggccccggaaaaggaccgccacccacacttgtgattacgcgggctgcggcaaaacctacacaaagagttcccatctcaaggcacacctgcgaacccacacaggtgagaaaccttaccactgtgactgggacggctgtggatggaaattcgcccgctcagatgaactgaccaggcactaccgtaaacacacggggcaccgcccgttccagtgccaaaaatgcgaccgagcattttccaggtcggaccacctcgccttacacatgaagaggcatttttaa

SEQ ID NO: 32 - DNA, 1320 bp, Homo sapiens
  source 1..1320: mol_type = genomic DNA
atgcccctcaacgttagcttcaccaacaggaactatgacctcgactacgactcggtgcagccgtatttctactgcgacgaggaggagaacttctaccagcagcagcagcagagcgagctgcagcccccggcgcccagcgaggatatctggaagaaattcgagctgctgcccaccccgcccctgtcccctagccgccgctccgggctctgctcgccctcctacgttgcggtcacacccttctcccttcggggagacaacgacggcggtggcgggagcttctccacggccgaccagctggagatggtgaccgagctgctgggaggagacatggtgaaccagagtttcatctgcgacccggacgacgagaccttcatcaaaaacatcatcatccaggactgtatgtggagcggcttctcggccgccgccaagctcgtctcagagaagctggcctcctaccaggctgcgcgcaaagacagcggcagcccgaaccccgcccgcggccacagcgtctgctccacctccagcttgtacctgcaggatctgagcgccgccgcctcagagtgcatcgacccctcggtggtcttcccctaccctctcaacgacagcagctcgcccaagtcctgcgcctcgcaagactccagcgccttctctccgtcctcggattctctgctctcctcgacggagtcctccccgcagggcagccccgagcccctggtgctccatgaggagacaccgcccaccaccagcagcgactctgaggaggaacaagaagatgaggaagaaatcgatgttgtttctgtggaaaagaggcaggctcctggcaaaaggtcagagtctggatcaccttctgctggaggccacagcaaacctcctcacagcccactggtcctcaagaggtgccacgtctccacacatcagcacaactacgcagcgcctccctccactcggaaggactatcctgctgccaagagggtcaagttggacagtgtcagagtcctgagacagatcagcaacaaccgaaaatgcaccagccccaggtcctcggacaccgaggagaatgtcaagaggcgaacacacaacgtcttggagcgccagaggaggaacgagctaaaacggagcttttttgccctgcgtgaccagatcccggagttggaaaacaatgaaaaggcccccaaggtagttatccttaaaaaagccacagcatacatcctgtccgtccaagcagaggagcaaaagctcatttctgaagaggacttgttgcggaaacgacgagaacagttgaaacacaaacttgaacagctacggaactcttgtgcgtaa

SEQ ID NO: 33 - protein, 562 aa, synthetic construct
  REGION 1..562: note = Primary structure of MeV/SeV F #2 chimeric F protein comprising C-terminal 33 aa truncated F protein of Measles virus Edmonston strain fused to C-terminal 42 aa of F protein of Sendai virus Z strain
MSIMGLKVNVSAIFMAVLLTLQTPTGQIHWGNLSKIGVVGIGSASYKVMTRSSHQSLVIKLMPNITLLNNCTRVEIAEYRRLLRTVLEPIRDALNAMTQNIRPVQSVASSRRHKRFAGVVLAGAALGVATAAQITAGIALHQSMLNSQAIDNLRASLETTNQAIEAIRQAGQEMILAVQGVQDYINNELIPSMNQLSCDLIGQKLGLKLLRYYTEILSLFGPSLRDPISAEISIQALSYALGGDINKVLEKLGYSGGDLLGILESRGIKARITHVDTESYFIVLSIAYPTLSEIKGVIVHRLEGVSYNIGSQEWYTTVPKYVATQGYLISNFDESSCTFMPEGTVCSQNALYPMSPLLQECLRGSTKSCARTLVSGSFGNRFILSQGNLIANCASILCKCYTTGTIINQDPDKILTYIAADHCPVVEVNGVTIQVGSRRYPDAVYLHRIDLGPPISLERLDVGTNLGNAIAKLEDAKELLESSDQILRSMKGLSSTSIVYILIAVCLGGLIGIPALICCCRLRRSMLMGNPDDRIPRDTYTLEPKIRHMYTNGGFDAMAEKR

SEQ ID NO: 34 - protein, 559 aa, synthetic construct
  REGION 1..559: note = Primary structure of MeV/SeV F #2 chimeric F protein comprising C-terminal 33 aa truncated F protein of Measles virus IC-B strain fused to C-terminal 42 aa of F protein of Sendai virus Z strain
MGLKVNVSAIFMAVLLTLQTPTGQIHWGNLSKIGVVGIGSASYKVMTRSSHQSLVIKLMPNITLLNNCTRVEIAEYRRLLRTVLEPIRDALNAMTQNIRPVQSVASSRRHKRFAGVVLAGAALGVATAAQITAGIALHQSMLNSQAIDNLRASLETTNQAIEAIRQAGQEMILAVQGVQDYINNELIPSMNQLSCDLIGQKLGLKLLRYYTEILSLFGPSLRDPISAEISIQALSYALGGDINKVLEKLGYSGGDLLGILESRGIKARITHVDTESYFIVLSIAYPTLSEIKGVIVHRLEGVSYNIGSQEWYTTVPKYVATQGYLISNFDESSCTFMPEGTVCSQNALYPMSPLLQECLRGSTKSCARTLVSGSFGNRFILSQGNLIANCASILCKCYTTGTIINQDPDKILTYIAADHCPVVEVNGVTIQVGSRRYPDAVYLHRIDLGPPISLERLDVGTNLGNAIAKLEDAKELLESSDQILRSMKGLSSTSIVYILIAVCLGGLIGIPALICCCRLRRSMLMGNPDDRIPRDTYTLEPKIRHMYTNGGFDAMAEKR

SEQ ID NO: 35 - protein, 619 aa, synthetic construct
  REGION 1..619: note = Primary structure of MeV/SeV H #1 chimeric H protein comprising N-terminal 60 aa of HN protein of Sendai virus Z strain fused to N-terminal 58 aa truncated H protein of Measles virus Edmonston strain
MDGDRGKRDSYWSTSPSGSTTKPASGWERSSKADTWLLILSFTQWALSIATVIICIIISARLHRAAIYTAEIHKSLSTNLDVTNSIEHQVKDVLTPLFKIIGDEVGLRTPQRFTDLVKFISDKIKFLNPDREYDFRDLTWCINPPERIKLDYDQYCADVAAEELMNALVNSTLLETRTTNQFLAVSKGNCSGPTTIRGQFSNMSLSLLDLYLGRGYNVSSIVTMTSQGMYGGTYLVEKPNLSSKRSELSQLSMYRVFEVGVIRNPGLGAPVFHMTNYLEQPVSNDLSNCMVALGELKLAALCHGEDSITIPYQGSGKGVSFQLVKLGVWKSPTDMQSWVPLSTDDPVIDRLYLSSHRGVIADNQAKWAVPTTRTDDKLRMETCFQQACKGKIQALCENPEWAPLKDNRIPSYGVLSVDLSLTVELKIKIASGFGPLITHGSGMDLYKSNHNNVYWLTIPPMKNLALGVINTLEWIPRFKVSPYLFNVPIKEAGEDCHAPTYLPAEVDGDVKLSSNLVILPGQDLQYVLATYDTSRVEHAVVYYVYSPSRSFSYFYPFRLPIKGVPIELQVECFTWDQKLWCRHFCVLADSESGGHITHSGMVGMGVSCTVTREDGTNRR

SEQ ID NO: 36 - protein, 68 aa, synthetic construct
  REGION 1..68: note = C-terminal part of F protein of Measles virus Edmonston strain
ILRSMKGLSSTSIVYILIAVCLGGLIGIPALICCCRGRCNKKGEQVGMSRPGLKPDLTGTSKSYVRSL

SEQ ID NO: 37 - protein, 38 aa, synthetic construct
  REGION 1..38: note = C-terminal part of MeV Fdel30 protein
ILRSMKGLSSTSIVYILIAVCLGGLIGIPALICCCRGR

SEQ ID NO: 38 - protein, 77 aa, synthetic construct
  REGION 1..77: note = C-terminal part of MeV/SeV F #2 protein
ILRSMKGLSSTSIVYILIAVCLGGLIGIPALICCCRLRRSMLMGNPDDRIPRDTYTLEPKIRHMYTNGGFDAMAEKR

SEQ ID NO: 39 - protein, 71 aa, synthetic construct
  REGION 1..71: note = C-terminal part of MeV/SeV F #1 protein
ILRSMKVITIIVVMVVILVVIIVIIIVLYRLRRSMLMGNPDDRIPRDTYTLEPKIRHMYTNGGFDAMAEKR

SEQ ID NO: 40 - protein, 71 aa, synthetic construct
  REGION 1..71: note = C-terminal part of Sendai virus F protein
YNSRETVITIIVVMVVILVVIIVIIIVLYRLRRSMLMGNPDDRIPRDTYTLEPKIRHMYTNGGFDAMAEKR

SEQ ID NO: 41 - protein, 64 aa, synthetic construct
  REGION 1..64: note = N-terminal part of Measles virus H protein
MSPQRDRINAFYKDNPHPKGSRIVINREHLMIDRPYVLLAVLFVMFLSLIGLLAIAGIRLHRAA

SEQ ID NO: 42 - protein, 46 aa, synthetic construct
  REGION 1..46: note = N-terminal part of MeV Hdel18 protein
MGSRIVINREHLMIDRPYVLLAVLFVMFLSLIGLLAIAGIRLHRAA

SEQ ID NO: 43 - protein, 65 aa, synthetic construct
  REGION 1..65: note = N-terminal part of MeV/SeV H #2 protein
MDGDRGKRDSYWSTSPSGSTTKPASGWERSSKADTPYVLLAVLFVMFLSLIGLLAIAGIRLHRAA

SEQ ID NO: 44 - protein, 66 aa, synthetic construct
  REGION 1..66: note = N-terminal part of MeV/SeV H #1 protein
MDGDRGKRDSYWSTSPSGSTTKPASGWERSSKADTWLLILSFTQWALSIATVIICIIISARLHRAA

SEQ ID NO: 45 - protein, 66 aa, synthetic construct
  REGION 1..66: note = N-terminal part of Sendai virus HN protein
MDGDRGKRDSYWSTSPSGSTTKPASGWERSSKADTWLLILSFTQWALSIATVIICIIISARQGYSM

SEQ ID NO: 46 - RNA, 51 nt, synthetic construct
  misc_feature 1..51: note = 5'-terminal sequence of F mRNA of Measles virus IC-B strain
  source 1..51: mol_type = other RNA
agaatcaagactcatccagtgtccatcatgggtctcaaggtgaacgtctct

SEQ ID NO: 47 - RNA, 51 nt, synthetic construct
  misc_feature 1..51: note = 5'-terminal sequence of F mRNA of Measles virus Edmonston strain
  source 1..51: mol_type = other RNA
agaatcaagactcatccaatgtccatcatgggtctcaaggtgaacgtctct

SEQ ID NO: 48 - protein, 8 aa, synthetic construct
  REGION 1..8: note = N-terminal part of F protein of Measles virus IC-B strain
MGLKVNVS

SEQ ID NO: 49 - protein, 11 aa, synthetic construct
  REGION 1..11: note = N-terminal part of F protein of Measles virus Edmonston strain
MSIMGLKVNVS

SEQ ID NO: 50 - DNA, 1860 bp, synthetic construct
  source 1..1860: mol_type = other DNA
  misc_feature 1..1860: note = cDNA encoding chimeric H protein comprising N-terminal 60 aa of HN protein of Sendai virus Z strain fused to N-terminal 58 aa truncated H protein of Measles virus IC-B strain
atggacggcgataggggcaagcgcgatagctactggtccacctctccaagcggctccaccacaaagccagcatccggatgggagcggagctccaaggcagacacctggctgctgatcctgtcctttacacagtgggccctgtctatcgccaccgtgatcatctgcatcatcatctccgcccggctgcacagagccgccatctatacagccgagatccacaagtctctgagcaccaacctggacgtgacaaattctatcgagcaccaggtgaaggatgtgctgacccctctgttcaagatcatcggcgacgaagtgggactgaggaccccacagcggttcaccgacctggtgaagttcatctccgataagatcaagtttctgaacccagatcgggagtacgacttcagagatctgacatggtgcatcaatccccctgagcggatcaagctggactacgatcagtattgtgccgacgtggccgccgaggagctgatgaacgccctggtgaatagcaccctgctggaggccagagccacaaaccagtttctggccgtgtccaagggcaattgttctggccccaccacaatcaggggccagttctccaacatgtccctgtctctgctggatctgtacctgtctcgcggctataacgtgagcagcatcgtgaccatgacatcccagggcatgtacggcggcacctatctggtgggcaagcccaacctgtcctctaagggcagcgagctgtcccagctgtctatgcacagggtgtttgaagtgggcgtgatcaggaaccctggactgggagccccagtgtttcacatgacaaattacttcgagcagcctgtgagcaacgatttttccaattgcatggtggccctgggagagctgaagttcgccgccctgtgccacagggaggactctatcaccatcccatatcagggcagcggcaagggcgtgtccttccagctggtgaagctgggcgtgtggaagagccccacagacatgagatcttgggtgcccctgagcaccgacgatcctgtgatcgatcggctgtacctgagctcccacagaggcgtgatcgcagacaaccaggcaaagtgggccgtgcctaccacaaggacagacgataagctgcgcatggagacctgctttcagcaggcctgtaagggcaagaaccaggccctgtgcgagaatcctgagtgggccccactgaaggataacaggatccctagctacggcgtgctgtctgtgaatctgagcctgacagtggagctgaagatcaagatcgcctctggcttcggcccactgatcacccacggcagcggcatggacctgtataagacaaatcacaacaacgtgtactggctgaccatcccacccatgaagaacctggccctgggcgtgatcaataccctggagtggatcccaaggtttaaggtgtcccccaacctgttcacagtgcctatcaaggaggcaggagaggattgtcacgcaccaacctacctgcctgcagaggtggacggcgatgtgaagctgtctagcaacctggtcatcctgccaggacaggacctgcagtacgtgctggccacctatgatacaagccgcgtggagcacgccgtggtgtactacgtgtactccccctcccggtctttcagctacttttatccattcagactgcccatcaagggcgtgcctatcgagctgcaggtggagtgctttacctgggataagaagctgtggtgcaggcacttctgcgtgctggcagactccgagtctggaggacacatcacacacagcggcatggtgggcatgggcgtgtcctgtaccgtgacacgcgaggacggcaccaaccggagatga

SEQ ID NO: 51 - protein, 619 aa, synthetic construct
  REGION 1..619: note = Primary structure of MeV(IC-B)/SeV H #1 chimeric H protein comprising N-terminal 60 aa of HN protein of Sendai virus Z strain fused to N-terminal 58 aa truncated H protein of Measles virus IC-B strain
MDGDRGKRDSYWSTSPSGSTTKPASGWERSSKADTWLLILSFTQWALSIATVIICIIISARLHRAAIYTAEIHKSLSTNLDVTNSIEHQVKDVLTPLFKIIGDEVGLRTPQRFTDLVKFISDKIKFLNPDREYDFRDLTWCINPPERIKLDYDQYCADVAAEELMNALVNSTLLEARATNQFLAVSKGNCSGPTTIRGQFSNMSLSLLDLYLSRGYNVSSIVTMTSQGMYGGTYLVGKPNLSSKGSELSQLSMHRVFEVGVIRNPGLGAPVFHMTNYFEQPVSNDFSNCMVALGELKFAALCHREDSITIPYQGSGKGVSFQLVKLGVWKSPTDMRSWVPLSTDDPVIDRLYLSSHRGVIADNQAKWAVPTTRTDDKLRMETCFQQACKGKNQALCENPEWAPLKDNRIPSYGVLSVNLSLTVELKIKIASGFGPLITHGSGMDLYKTNHNNVYWLTIPPMKNLALGVINTLEWIPRFKVSPNLFTVPIKEAGEDCHAPTYLPAEVDGDVKLSSNLVILPGQDLQYVLATYDTSRVEHAVVYYVYSPSRSFSYFYPFRLPIKGVPIELQVECFTWDKKLWCRHFCVLADSESGGHITHSGMVGMGVSCTVTREDGTNRR